European Patent Application EP 4 268 823 A1, published November 1, 2023. Title: COMPOUND FOR TREATING NEUROINFLAMMATION. Applicant: Universitätsklinikum Hamburg-Eppendorf. The sequence listing filed with the application follows.

SEQUENCE LISTING (8 sequences)

SEQ ID NO: 1 - DNA, 3804 bp, Homo sapiens
atgcggggtctaccgagagggagggggttgatgcgggcccgggggaggggtcgtgcggcccctccgggcagccgaggccgcggaaggggggggccccacagaggaagaggtaggccccggagcctactctctcttcccagggcccaggcatcctggaccccccaactctctactgggctgaccagccctcctgtcccttgtctcccctcccagggggaggcccccgctgagatgggggcgctgctgctggagaaggaaaccagaggagccaccgagagagttcatggctctttgggggacacccctcgtagtgaagaaaccctgcccaaggccacccccgactccctggagcctgctggcccctcatctccagcctctgtcactgtcactgttggtgatgagggggctgacacccctgtaggggctacaccactcattggggatgaatctgagaatcttgagggagatggggacctccgtgggggccggatcctgctgggccatgccacaaagtcattcccctcttcccccagcaaggggggttcctgtcctagccgggccaagatgtcaatgacaggggcgggaaaatcacctccatctgtccagagtttggctatgaggctactgagtatgccaggagcccagggagctgcagcagcagggtctgaaccccctccagccaccacgagcccagagggacagcccaaggtccaccgagcccgcaaaaccatgtccaaaccaggaaatggacagcccccggtccctgagaagcggccccctgaaatacagcatttccgcatgagtgatgatgtccactcactgggaaaggtgacctcagatctggccaaaaggaggaagctgaactcaggaggtggcctgtcagaggagttaggttctgcccggcgttcaggagaagtgaccctgacgaaaggggaccccgggtccctggaggagtgggagacggtggtgggtgatgacttcagtctctactatgattcctactctgtggatgagcgcgtggactccgacagcaagtctgaagttgaagctctaactgaacaactaagtgaagaggaggaggaggaagaggaggaagaagaagaagaggaagaggaggaggaagaggaagaagaagaggaagatgaggagtcagggaatcagtcagataggagtggttccagtggccggcgcaaggccaagaagaaatggcgaaaagacagcccatgggtgaagccgtctcggaaacggcgcaagcgggagcctccgcgggccaaggagccacgaggagtgaatggtgtgggctcctcaggccccagtgagtacatggaggtccctctggggtccctggagctgcccagcgaggggaccctctcccccaaccacgctggggtgtccaatgacacatcttcgctggagacagagcgagggtttgaggagttgcccctgtgcagctgccgcatggaggcacccaagattgaccgcatcagcgagagggcggggcacaagtgcatggccactgagagtgtggacggagagctgtcaggctgcaatgccgccatcctcaagcgggagaccatgaggccatccagccgtgtggccctgatggtgctctgtgagacccaccgcgcccgcatggtcaaacaccactgctgcccgggctgcggctacttctgcacggcgggcaccttcctggagtgccaccctgacttccgtgtggcccaccgcttccacaaggcctgtgtgtctcagctgaatgggatggtcttctgtccccactgtggggaggatgcttctgaagctcaagaggtgaccatcccccggggtgacggggtgaccccaccggccggcactgcagctcctgcacccccacccctgtcccaggatgtccccgggagagcagacacttctcagcccagtgcccggatgcgagggcatggggaaccccggcgcccgccctgcgatcccctggctgacaccattgacagctcagggccctccctgaccctgcccaatgggggctgcctttcagccgtggggctgccactggggccaggccgggaggccctggaaaaggccctggtcatccaggagtcagagaggcggaagaagctccgtttccaccctcggcagttgtacctgtccgtgaagcagggcgagctgcagaaggtgatcctgatgctgttggacaacctggaccccaacttccagagcgaccagcagagcaagcgcacgcccctgcatgcagccgcccagaagggctccgtggagatctgccatgtgctgctgcaggctggagccaacataaatgcagtggacaaacagcagcggacgccactgatggaggccgtggtgaacaaccacctggaggtagcccgttacatggtgcagcgtggtggctgtgtctatagcaaggaggaggacggttccacctgcctccaccacgcagccaaaatcgggaacttggagatggtcagcctgctgctgagcacaggacaggtggacgtcaacgcccaggacagtggggggtggacgcccatcatctgggctgcagagcacaagcacatcgaggtgatccgcatgctactgacgcggggcgccgacgtcaccctcactgacaacgaggagaacatctgcctgcactgggcctccttcacgggcagcgccgccatcgccgaagtccttctgaatgcgcgctgtgacctccatgctgtcaactaccatggggacacccccctgcacatcgcagctcgggagagctaccatgactgcgtgctgttattcctgtcacgtggggccaaccctgagctgcggaacaaagagggggacacagcatgggacctgactcccgagcgctccgacgtgtggtttgcgcttcaactcaaccgcaagctccgacttggggtgggaaatcgggccatccgcacagagaagatcatctgccgggacgtggctcggggctatgagaacgtgcccattccctgtgtcaacggtgtggatggggagccctgccctgaggattacaagtacatctcagagaactgcgagacgtccaccatgaacatcgatcgcaacatcacccacctgcagcactgcacgtgtgtggacgactgctctagctccaactgcctgtgcggccagctcagcatccggtgctggtatgacaaggatgggcgattgctccaggaatttaacaagattgagcctccgctgattttcgagtgtaaccaggcgtgctcatgctggagaaactgcaagaaccgggtcgtacagagtggcatcaaggtgcggctacagctctaccgaacagccaagatgggctggggggtccgcgccctgcagaccatcccacaggggaccttcatctgcgagtatgtcggggagctgatctctgatgctgaggctgatgtgagagaggatgattcttacctcttcgacttagacaacaaggatggagaggtgtactgcatagatgcccgttactatggcaacatcagccgcttcatcaaccacctgtgtgaccccaacatcattcccgtccgggtcttcatgctgcaccaagacctgcgatttccacgcatcgccttcttcagttcccgagacatccggactggggaggagctagggtttgactatggcgaccgcttctgggacatcaaaagcaaatatttcacctgccaatgtggctctgagaagtgcaagcactcagccgaagccattgccctggagcagagccgtctggcccgcctggacccacaccctgagctgctgcccgagctcggctccctgccccctgtcaacacatga

SEQ ID NO: 2 - DNA, 3633 bp, Homo sapiens
atggcggcggcggcgggagctgcagcggcggcggccgccgagggggaggcccccgctgagatgggggcgctgctgctggagaaggaaaccagaggagccaccgagagagttcatggctctttgggggacacccctcgtagtgaagaaaccctgcccaaggccacccccgactccctggagcctgctggcccctcatctccagcctctgtcactgtcactgttggtgatgagggggctgacacccctgtaggggctacaccactcattggggatgaatctgagaatcttgagggagatggggacctccgtgggggccggatcctgctgggccatgccacaaagtcattcccctcttcccccagcaaggggggttcctgtcctagccgggccaagatgtcaatgacaggggcgggaaaatcacctccatctgtccagagtttggctatgaggctactgagtatgccaggagcccagggagctgcagcagcagggtctgaaccccctccagccaccacgagcccagagggacagcccaaggtccaccgagcccgcaaaaccatgtccaaaccaggaaatggacagcccccggtccctgagaagcggccccctgaaatacagcatttccgcatgagtgatgatgtccactcactgggaaaggtgacctcagatctggccaaaaggaggaagctgaactcaggaggtggcctgtcagaggagttaggttctgcccggcgttcaggagaagtgaccctgacgaaaggggaccccgggtccctggaggagtgggagacggtggtgggtgatgacttcagtctctactatgattcctactctgtggatgagcgcgtggactccgacagcaagtctgaagttgaagctctaactgaacaactaagtgaagaggaggaggaggaagaggaggaagaagaagaagaggaagaggaggaggaagaggaagaagaagaggaagatgaggagtcagggaatcagtcagataggagtggttccagtggccggcgcaaggccaagaagaaatggcgaaaagacagcccatgggtgaagccgtctcggaaacggcgcaagcgggagcctccgcgggccaaggagccacgaggagtgaatggtgtgggctcctcaggccccagtgagtacatggaggtccctctggggtccctggagctgcccagcgaggggaccctctcccccaaccacgctggggtgtccaatgacacatcttcgctggagacagagcgagggtttgaggagttgcccctgtgcagctgccgcatggaggcacccaagattgaccgcatcagcgagagggcggggcacaagtgcatggccactgagagtgtggacggagagctgtcaggctgcaatgccgccatcctcaagcgggagaccatgaggccatccagccgtgtggccctgatggtgctctgtgagacccaccgcgcccgcatggtcaaacaccactgctgcccgggctgcggctacttctgcacggcgggcaccttcctggagtgccaccctgacttccgtgtggcccaccgcttccacaaggcctgtgtgtctcagctgaatgggatggtcttctgtccccactgtggggaggatgcttctgaagctcaagaggtgaccatcccccggggtgacggggtgaccccaccggccggcactgcagctcctgcacccccacccctgtcccaggatgtccccgggagagcagacacttctcagcccagtgcccggatgcgagggcatggggaaccccggcgcccgccctgcgatcccctggctgacaccattgacagctcagggccctccctgaccctgcccaatgggggctgcctttcagccgtggggctgccactggggccaggccgggaggccctggaaaaggccctggtcatccaggagtcagagaggcggaagaagctccgtttccaccctcggcagttgtacctgtccgtgaagcagggcgagctgcagaaggtgatcctgatgctgttggacaacctggaccccaacttccagagcgaccagcagagcaagcgcacgcccctgcatgcagccgcccagaagggctccgtggagatctgccatgtgctgctgcaggctggagccaacataaatgcagtggacaaacagcagcggacgccactgatggaggccgtggtgaacaaccacctggaggtagcccgttacatggtgcagcgtggtggctgtgtctatagcaaggaggaggacggttccacctgcctccaccacgcagccaaaatcgggaacttggagatggtcagcctgctgctgagcacaggacaggtggacgtcaacgcccaggacagtggggggtggacgcccatcatctgggctgcagagcacaagcacatcgaggtgatccgcatgctactgacgcggggcgccgacgtcaccctcactgacaacgaggagaacatctgcctgcactgggcctccttcacgggcagcgccgccatcgccgaagtccttctgaatgcgcgctgtgacctccatgctgtcaactaccatggggacacccccctgcacatcgcagctcgggagagctaccatgactgcgtgctgttattcctgtcacgtggggccaaccctgagctgcggaacaaagagggggacacagcatgggacctgactcccgagcgctccgacgtgtggtttgcgcttcaactcaaccgcaagctccgacttggggtgggaaatcgggccatccgcacagagaagatcatctgccgggacgtggctcggggctatgagaacgtgcccattccctgtgtcaacggtgtggatggggagccctgccctgaggattacaagtacatctcagagaactgcgagacgtccaccatgaacatcgatcgcaacatcacccacctgcagcactgcacgtgtgtggacgactgctctagctccaactgcctgtgcggccagctcagcatccggtgctggtatgacaaggatgggcgattgctccaggaatttaacaagattgagcctccgctgattttcgagtgtaaccaggcgtgctcatgctggagaaactgcaagaaccgggtcgtacagagtggcatcaaggtgcggctacagctctaccgaacagccaagatgggctggggggtccgcgccctgcagaccatcccacaggggaccttcatctgcgagtatgtcggggagctgatctctgatgctgaggctgatgtgagagaggatgattcttacctcttcgacttagacaacaaggatggagaggtgtactgcatagatgcccgttactatggcaacatcagccgcttcatcaaccacctgtgtgaccccaacatcattcccgtccgggtcttcatgctgcaccaagacctgcgatttccacgcatcgccttcttcagttcccgagacatccggactggggaggagctagggtttgactatggcgaccgcttctgggacatcaaaagcaaatatttcacctgccaatgtggctctgagaagtgcaagcactcagccgaagccattgccctggagcagagccgtctggcccgcctggacccacaccctgagctgctgcccgagctcggctccctgccccctgtcaacacatga

SEQ ID NO: 3 - DNA, 3531 bp, Homo sapiens
atggcggcggcggcgggagctgcagcggcggcggccgccgagggggaggcccccgctgagatgggggcgctgctgctggagaaggaaaccagaggagccaccgagagagttcatggctctttgggggacacccctcgtagtgaagaaaccctgcccaaggccacccccgactccctggagcctgctggcccctcatctccagcctctgtcactgtcactgttggtgatgagggggctgacacccctgtaggggctacaccactcattggggatgaatctgagaatcttgagggagatggggacctccgtgggggccggatcctgctgggccatgccacaaagtcattcccctcttcccccagcaaggggggttcctgtcctagccgggccaagatgtcaatgacaggggcgggaaaatcacctccatctgtccagagtttggctatgaggctactgagtatgccaggagcccagggagctgcagcagcagggtctgaaccccctccagccaccacgagcccagagggacagcccaaggtccaccgagcccgcaaaaccatgtccaaaccaggaaatggacagcccccggtccctgagaagcggccccctgaaatacagcatttccgcatgagtgatgatgtccactcactgggaaaggtgacctcagatctggccaaaaggaggaagctgaactcaggaggtggcctgtcagaggagttaggttctgcccggcgttcaggagaagtgaccctgacgaaaggggaccccgggtccctggaggagtgggagacggtggtgggtgatgacttcagtctctactatgattcctactctgtggatgagcgcgtggactccgacagcaagtctgaagttgaagctctaactgaacaactaagtgaagaggaggaggaggaagaggaggaagaagaagaagaggaagaggaggaggaagaggaagaagaagaggaagatgaggagtcagggaatcagtcagataggagtggttccagtggccggcgcaaggccaagaagaaatggcgaaaagacagcccatgggtgaagccgtctcggaaacggcgcaagcgggagcctccgcgggccaaggagccacgaggggtgtccaatgacacatcttcgctggagacagagcgagggtttgaggagttgcccctgtgcagctgccgcatggaggcacccaagattgaccgcatcagcgagagggcggggcacaagtgcatggccactgagagtgtggacggagagctgtcaggctgcaatgccgccatcctcaagcgggagaccatgaggccatccagccgtgtggccctgatggtgctctgtgagacccaccgcgcccgcatggtcaaacaccactgctgcccgggctgcggctacttctgcacggcgggcaccttcctggagtgccaccctgacttccgtgtggcccaccgcttccacaaggcctgtgtgtctcagctgaatgggatggtcttctgtccccactgtggggaggatgcttctgaagctcaagaggtgaccatcccccggggtgacggggtgaccccaccggccggcactgcagctcctgcacccccacccctgtcccaggatgtccccgggagagcagacacttctcagcccagtgcccggatgcgagggcatggggaaccccggcgcccgccctgcgatcccctggctgacaccattgacagctcagggccctccctgaccctgcccaatgggggctgcctttcagccgtggggctgccactggggccaggccgggaggccctggaaaaggccctggtcatccaggagtcagagaggcggaagaagctccgtttccaccctcggcagttgtacctgtccgtgaagcagggcgagctgcagaaggtgatcctgatgctgttggacaacctggaccccaacttccagagcgaccagcagagcaagcgcacgcccctgcatgcagccgcccagaagggctccgtggagatctgccatgtgctgctgcaggctggagccaacataaatgcagtggacaaacagcagcggacgccactgatggaggccgtggtgaacaaccacctggaggtagcccgttacatggtgcagcgtggtggctgtgtctatagcaaggaggaggacggttccacctgcctccaccacgcagccaaaatcgggaacttggagatggtcagcctgctgctgagcacaggacaggtggacgtcaacgcccaggacagtggggggtggacgcccatcatctgggctgcagagcacaagcacatcgaggtgatccgcatgctactgacgcggggcgccgacgtcaccctcactgacaacgaggagaacatctgcctgcactgggcctccttcacgggcagcgccgccatcgccgaagtccttctgaatgcgcgctgtgacctccatgctgtcaactaccatggggacacccccctgcacatcgcagctcgggagagctaccatgactgcgtgctgttattcctgtcacgtggggccaaccctgagctgcggaacaaagagggggacacagcatgggacctgactcccgagcgctccgacgtgtggtttgcgcttcaactcaaccgcaagctccgacttggggtgggaaatcgggccatccgcacagagaagatcatctgccgggacgtggctcggggctatgagaacgtgcccattccctgtgtcaacggtgtggatggggagccctgccctgaggattacaagtacatctcagagaactgcgagacgtccaccatgaacatcgatcgcaacatcacccacctgcagcactgcacgtgtgtggacgactgctctagctccaactgcctgtgcggccagctcagcatccggtgctggtatgacaaggatgggcgattgctccaggaatttaacaagattgagcctccgctgattttcgagtgtaaccaggcgtgctcatgctggagaaactgcaagaaccgggtcgtacagagtggcatcaaggtgcggctacagctctaccgaacagccaagatgggctggggggtccgcgccctgcagaccatcccacaggggaccttcatctgcgagtatgtcggggagctgatctctgatgctgaggctgatgtgagagaggatgattcttacctcttcgacttagacaacaaggatggagaggtgtactgcatagatgcccgttactatggcaacatcagccgcttcatcaaccacctgtgtgaccccaacatcattcccgtccgggtcttcatgctgcaccaagacctgcgatttccacgcatcgccttcttcagttcccgagacatccggactggggaggagctagggtttgactatggcgaccgcttctgggacatcaaaagcaaatatttcacctgccaatgtggctctgagaagtgcaagcactcagccgaagccattgccctggagcagagccgtctggcccgcctggacccacaccctgagctgctgcccgagctcggctccctgccccctgtcaacacatga

SEQ ID NO: 4 - DNA, 3702 bp, Homo sapiens
atgcggggtctaccgagagggagggggttgatgcgggcccgggggaggggtcgtgcggcccctccgggcagccgaggccgcggaaggggggggccccacagaggaagaggtaggccccggagcctactctctcttcccagggcccaggcatcctggaccccccaactctctactgggctgaccagccctcctgtcccttgtctcccctcccagggggaggcccccgctgagatgggggcgctgctgctggagaaggaaaccagaggagccaccgagagagttcatggctctttgggggacacccctcgtagtgaagaaaccctgcccaaggccacccccgactccctggagcctgctggcccctcatctccagcctctgtcactgtcactgttggtgatgagggggctgacacccctgtaggggctacaccactcattggggatgaatctgagaatcttgagggagatggggacctccgtgggggccggatcctgctgggccatgccacaaagtcattcccctcttcccccagcaaggggggttcctgtcctagccgggccaagatgtcaatgacaggggcgggaaaatcacctccatctgtccagagtttggctatgaggctactgagtatgccaggagcccagggagctgcagcagcagggtctgaaccccctccagccaccacgagcccagagggacagcccaaggtccaccgagcccgcaaaaccatgtccaaaccaggaaatggacagcccccggtccctgagaagcggccccctgaaatacagcatttccgcatgagtgatgatgtccactcactgggaaaggtgacctcagatctggccaaaaggaggaagctgaactcaggaggtggcctgtcagaggagttaggttctgcccggcgttcaggagaagtgaccctgacgaaaggggaccccgggtccctggaggagtgggagacggtggtgggtgatgacttcagtctctactatgattcctactctgtggatgagcgcgtggactccgacagcaagtctgaagttgaagctctaactgaacaactaagtgaagaggaggaggaggaagaggaggaagaagaagaagaggaagaggaggaggaagaggaagaagaagaggaagatgaggagtcagggaatcagtcagataggagtggttccagtggccggcgcaaggccaagaagaaatggcgaaaagacagcccatgggtgaagccgtctcggaaacggcgcaagcgggagcctccgcgggccaaggagccacgaggggtgtccaatgacacatcttcgctggagacagagcgagggtttgaggagttgcccctgtgcagctgccgcatggaggcacccaagattgaccgcatcagcgagagggcggggcacaagtgcatggccactgagagtgtggacggagagctgtcaggctgcaatgccgccatcctcaagcgggagaccatgaggccatccagccgtgtggccctgatggtgctctgtgagacccaccgcgcccgcatggtcaaacaccactgctgcccgggctgcggctacttctgcacggcgggcaccttcctggagtgccaccctgacttccgtgtggcccaccgcttccacaaggcctgtgtgtctcagctgaatgggatggtcttctgtccccactgtggggaggatgcttctgaagctcaagaggtgaccatcccccggggtgacggggtgaccccaccggccggcactgcagctcctgcacccccacccctgtcccaggatgtccccgggagagcagacacttctcagcccagtgcccggatgcgagggcatggggaaccccggcgcccgccctgcgatcccctggctgacaccattgacagctcagggccctccctgaccctgcccaatgggggctgcctttcagccgtggggctgccactggggccaggccgggaggccctggaaaaggccctggtcatccaggagtcagagaggcggaagaagctccgtttccaccctcggcagttgtacctgtccgtgaagcagggcgagctgcagaaggtgatcctgatgctgttggacaacctggaccccaacttccagagcgaccagcagagcaagcgcacgcccctgcatgcagccgcccagaagggctccgtggagatctgccatgtgctgctgcaggctggagccaacataaatgcagtggacaaacagcagcggacgccactgatggaggccgtggtgaacaaccacctggaggtagcccgttacatggtgcagcgtggtggctgtgtctatagcaaggaggaggacggttccacctgcctccaccacgcagccaaaatcgggaacttggagatggtcagcctgctgctgagcacaggacaggtggacgtcaacgcccaggacagtggggggtggacgcccatcatctgggctgcagagcacaagcacatcgaggtgatccgcatgctactgacgcggggcgccgacgtcaccctcactgacaacgaggagaacatctgcctgcactgggcctccttcacgggcagcgccgccatcgccgaagtccttctgaatgcgcgctgtgacctccatgctgtcaactaccatggggacacccccctgcacatcgcagctcgggagagctaccatgactgcgtgctgttattcctgtcacgtggggccaaccctgagctgcggaacaaagagggggacacagcatgggacctgactcccgagcgctccgacgtgtggtttgcgcttcaactcaaccgcaagctccgacttggggtgggaaatcgggccatccgcacagagaagatcatctgccgggacgtggctcggggctatgagaacgtgcccattccctgtgtcaacggtgtggatggggagccctgccctgaggattacaagtacatctcagagaactgcgagacgtccaccatgaacatcgatcgcaacatcacccacctgcagcactgcacgtgtgtggacgactgctctagctccaactgcctgtgcggccagctcagcatccggtgctggtatgacaaggatgggcgattgctccaggaatttaacaagattgagcctccgctgattttcgagtgtaaccaggcgtgctcatgctggagaaactgcaagaaccgggtcgtacagagtggcatcaaggtgcggctacagctctaccgaacagccaagatgggctggggggtccgcgccctgcagaccatcccacaggggaccttcatctgcgagtatgtcggggagctgatctctgatgctgaggctgatgtgagagaggatgattcttacctcttcgacttagacaacaaggatggagaggtgtactgcatagatgcccgttactatggcaacatcagccgcttcatcaaccacctgtgtgaccccaacatcattcccgtccgggtcttcatgctgcaccaagacctgcgatttccacgcatcgccttcttcagttcccgagacatccggactggggaggagctagggtttgactatggcgaccgcttctgggacatcaaaagcaaatatttcacctgccaatgtggctctgagaagtgcaagcactcagccgaagccattgccctggagcagagccgtctggcccgcctggacccacaccctgagctgctgcccgagctcggctccctgccccctgtcaacacatga

SEQ ID NO: 5 - protein, 1267 aa, Homo sapiens
MRGLPRGRGLMRARGRGRAAPPGSRGRGRGGPHRGRGRPRSLLSLPRAQASWTPQLSTGLTSPPVPCLPSQGEAPAEMGALLLEKETRGATERVHGSLGDTPRSEETLPKATPDSLEPAGPSSPASVTVTVGDEGADTPVGATPLIGDESENLEGDGDLRGGRILLGHATKSFPSSPSKGGSCPSRAKMSMTGAGKSPPSVQSLAMRLLSMPGAQGAAAAGSEPPPATTSPEGQPKVHRARKTMSKPGNGQPPVPEKRPPEIQHFRMSDDVHSLGKVTSDLAKRRKLNSGGGLSEELGSARRSGEVTLTKGDPGSLEEWETVVGDDFSLYYDSYSVDERVDSDSKSEVEALTEQLSEEEEEEEEEEEEEEEEEEEEEEEEDEESGNQSDRSGSSGRRKAKKKWRKDSPWVKPSRKRRKREPPRAKEPRGVNGVGSSGPSEYMEVPLGSLELPSEGTLSPNHAGVSNDTSSLETERGFEELPLCSCRMEAPKIDRISERAGHKCMATESVDGELSGCNAAILKRETMRPSSRVALMVLCETHRARMVKHHCCPGCGYFCTAGTFLECHPDFRVAHRFHKACVSQLNGMVFCPHCGEDASEAQEVTIPRGDGVTPPAGTAAPAPPPLSQDVPGRADTSQPSARMRGHGEPRRPPCDPLADTIDSSGPSLTLPNGGCLSAVGLPLGPGREALEKALVIQESERRKKLRFHPRQLYLSVKQGELQKVILMLLDNLDPNFQSDQQSKRTPLHAAAQKGSVEICHVLLQAGANINAVDKQQRTPLMEAVVNNHLEVARYMVQRGGCVYSKEEDGSTCLHHAAKIGNLEMVSLLLSTGQVDVNAQDSGGWTPIIWAAEHKHIEVIRMLLTRGADVTLTDNEENICLHWASFTGSAAIAEVLLNARCDLHAVNYHGDTPLHIAARESYHDCVLLFLSRGANPELRNKEGDTAWDLTPERSDVWFALQLNRKLRLGVGNRAIRTEKIICRDVARGYENVPIPCVNGVDGEPCPEDYKYISENCETSTMNIDRNITHLQHCTCVDDCSSSNCLCGQLSIRCWYDKDGRLLQEFNKIEPPLIFECNQACSCWRNCKNRVVQSGIKVRLQLYRTAKMGWGVRALQTIPQGTFICEYVGELISDAEADVREDDSYLFDLDNKDGEVYCIDARYYGNISRFINHLCDPNIIPVRVFMLHQDLRFPRIAFFSSRDIRTGEELGFDYGDRFWDIKSKYFTCQCGSEKCKHSAEAIALEQSRLARLDPHPELLPELGSLPPVNT

SEQ ID NO: 6 - protein, 1210 aa, Homo sapiens
MAAAAGAAAAAAAEGEAPAEMGALLLEKETRGATERVHGSLGDTPRSEETLPKATPDSLEPAGPSSPASVTVTVGDEGADTPVGATPLIGDESENLEGDGDLRGGRILLGHATKSFPSSPSKGGSCPSRAKMSMTGAGKSPPSVQSLAMRLLSMPGAQGAAAAGSEPPPATTSPEGQPKVHRARKTMSKPGNGQPPVPEKRPPEIQHFRMSDDVHSLGKVTSDLAKRRKLNSGGGLSEELGSARRSGEVTLTKGDPGSLEEWETVVGDDFSLYYDSYSVDERVDSDSKSEVEALTEQLSEEEEEEEEEEEEEEEEEEEEEEEEDEESGNQSDRSGSSGRRKAKKKWRKDSPWVKPSRKRRKREPPRAKEPRGVNGVGSSGPSEYMEVPLGSLELPSEGTLSPNHAGVSNDTSSLETERGFEELPLCSCRMEAPKIDRISERAGHKCMATESVDGELSGCNAAILKRETMRPSSRVALMVLCETHRARMVKHHCCPGCGYFCTAGTFLECHPDFRVAHRFHKACVSQLNGMVFCPHCGEDASEAQEVTIPRGDGVTPPAGTAAPAPPPLSQDVPGRADTSQPSARMRGHGEPRRPPCDPLADTIDSSGPSLTLPNGGCLSAVGLPLGPGREALEKALVIQESERRKKLRFHPRQLYLSVKQGELQKVILMLLDNLDPNFQSDQQSKRTPLHAAAQKGSVEICHVLLQAGANINAVDKQQRTPLMEAVVNNHLEVARYMVQRGGCVYSKEEDGSTCLHHAAKIGNLEMVSLLLSTGQVDVNAQDSGGWTPIIWAAEHKHIEVIRMLLTRGADVTLTDNEENICLHWASFTGSAAIAEVLLNARCDLHAVNYHGDTPLHIAARESYHDCVLLFLSRGANPELRNKEGDTAWDLTPERSDVWFALQLNRKLRLGVGNRAIRTEKIICRDVARGYENVPIPCVNGVDGEPCPEDYKYISENCETSTMNIDRNITHLQHCTCVDDCSSSNCLCGQLSIRCWYDKDGRLLQEFNKIEPPLIFECNQACSCWRNCKNRVVQSGIKVRLQLYRTAKMGWGVRALQTIPQGTFICEYVGELISDAEADVREDDSYLFDLDNKDGEVYCIDARYYGNISRFINHLCDPNIIPVRVFMLHQDLRFPRIAFFSSRDIRTGEELGFDYGDRFWDIKSKYFTCQCGSEKCKHSAEAIALEQSRLARLDPHPELLPELGSLPPVNT

SEQ ID NO: 7 - protein, 1176 aa, Homo sapiens
MAAAAGAAAAAAAEGEAPAEMGALLLEKETRGATERVHGSLGDTPRSEETLPKATPDSLEPAGPSSPASVTVTVGDEGADTPVGATPLIGDESENLEGDGDLRGGRILLGHATKSFPSSPSKGGSCPSRAKMSMTGAGKSPPSVQSLAMRLLSMPGAQGAAAAGSEPPPATTSPEGQPKVHRARKTMSKPGNGQPPVPEKRPPEIQHFRMSDDVHSLGKVTSDLAKRRKLNSGGGLSEELGSARRSGEVTLTKGDPGSLEEWETVVGDDFSLYYDSYSVDERVDSDSKSEVEALTEQLSEEEEEEEEEEEEEEEEEEEEEEEEDEESGNQSDRSGSSGRRKAKKKWRKDSPWVKPSRKRRKREPPRAKEPRGVSNDTSSLETERGFEELPLCSCRMEAPKIDRISERAGHKCMATESVDGELSGCNAAILKRETMRPSSRVALMVLCETHRARMVKHHCCPGCGYFCTAGTFLECHPDFRVAHRFHKACVSQLNGMVFCPHCGEDASEAQEVTIPRGDGVTPPAGTAAPAPPPLSQDVPGRADTSQPSARMRGHGEPRRPPCDPLADTIDSSGPSLTLPNGGCLSAVGLPLGPGREALEKALVIQESERRKKLRFHPRQLYLSVKQGELQKVILMLLDNLDPNFQSDQQSKRTPLHAAAQKGSVEICHVLLQAGANINAVDKQQRTPLMEAVVNNHLEVARYMVQRGGCVYSKEEDGSTCLHHAAKIGNLEMVSLLLSTGQVDVNAQDSGGWTPIIWAAEHKHIEVIRMLLTRGADVTLTDNEENICLHWASFTGSAAIAEVLLNARCDLHAVNYHGDTPLHIAARESYHDCVLLFLSRGANPELRNKEGDTAWDLTPERSDVWFALQLNRKLRLGVGNRAIRTEKIICRDVARGYENVPIPCVNGVDGEPCPEDYKYISENCETSTMNIDRNITHLQHCTCVDDCSSSNCLCGQLSIRCWYDKDGRLLQEFNKIEPPLIFECNQACSCWRNCKNRVVQSGIKVRLQLYRTAKMGWGVRALQTIPQGTFICEYVGELISDAEADVREDDSYLFDLDNKDGEVYCIDARYYGNISRFINHLCDPNIIPVRVFMLHQDLRFPRIAFFSSRDIRTGEELGFDYGDRFWDIKSKYFTCQCGSEKCKHSAEAIALEQSRLARLDPHPELLPELGSLPPVNT

SEQ ID NO: 8 - protein, 1233 aa, Homo sapiens
MRGLPRGRGLMRARGRGRAAPPGSRGRGRGGPHRGRGRPRSLLSLPRAQASWTPQLSTGLTSPPVPCLPSQGEAPAEMGALLLEKETRGATERVHGSLGDTPRSEETLPKATPDSLEPAGPSSPASVTVTVGDEGADTPVGATPLIGDESENLEGDGDLRGGRILLGHATKSFPSSPSKGGSCPSRAKMSMTGAGKSPPSVQSLAMRLLSMPGAQGAAAAGSEPPPATTSPEGQPKVHRARKTMSKPGNGQPPVPEKRPPEIQHFRMSDDVHSLGKVTSDLAKRRKLNSGGGLSEELGSARRSGEVTLTKGDPGSLEEWETVVGDDFSLYYDSYSVDERVDSDSKSEVEALTEQLSEEEEEEEEEEEEEEEEEEEEEEEEDEESGNQSDRSGSSGRRKAKKKWRKDSPWVKPSRKRRKREPPRAKEPRGVSNDTSSLETERGFEELPLCSCRMEAPKIDRISERAGHKCMATESVDGELSGCNAAILKRETMRPSSRVALMVLCETHRARMVKHHCCPGCGYFCTAGTFLECHPDFRVAHRFHKACVSQLNGMVFCPHCGEDASEAQEVTIPRGDGVTPPAGTAAPAPPPLSQDVPGRADTSQPSARMRGHGEPRRPPCDPLADTIDSSGPSLTLPNGGCLSAVGLPLGPGREALEKALVIQESERRKKLRFHPRQLYLSVKQGELQKVILMLLDNLDPNFQSDQQSKRTPLHAAAQKGSVEICHVLLQAGANINAVDKQQRTPLMEAVVNNHLEVARYMVQRGGCVYSKEEDGSTCLHHAAKIGNLEMVSLLLSTGQVDVNAQDSGGWTPIIWAAEHKHIEVIRMLLTRGADVTLTDNEENICLHWASFTGSAAIAEVLLNARCDLHAVNYHGDTPLHIAARESYHDCVLLFLSRGANPELRNKEGDTAWDLTPERSDVWFALQLNRKLRLGVGNRAIRTEKIICRDVARGYENVPIPCVNGVDGEPCPEDYKYISENCETSTMNIDRNITHLQHCTCVDDCSSSNCLCGQLSIRCWYDKDGRLLQEFNKIEPPLIFECNQACSCWRNCKNRVVQSGIKVRLQLYRTAKMGWGVRALQTIPQGTFICEYVGELISDAEADVREDDSYLFDLDNKDGEVYCIDARYYGNISRFINHLCDPNIIPVRVFMLHQDLRFPRIAFFSSRDIRTGEELGFDYGDRFWDIKSKYFTCQCGSEKCKHSAEAIALEQSRLARLDPHPELLPELGSLPPVNT